European Patent Application EP 4 737 471 A1, published May 6, 2026. Title: METHODS FOR THE C-TERMINAL MODIFICATION OF (POLY)PEPTIDES. Applicant: Numaferm GmbH. The sequence listing filed with the application follows.

SEQUENCE LISTING (6 sequences)

SEQ ID NO: 1 - protein, 4 aa, synthetic construct
FYGF

SEQ ID NO: 2 - protein, 4 aa, synthetic construct
FGYF

SEQ ID NO: 3 - protein, 7 aa, synthetic construct
CHHHHHH

SEQ ID NO: 4 - protein, 11 aa, synthetic construct
CGGGGSGGGGS

SEQ ID NO: 5 - protein, 6 aa, synthetic construct
PNDKYE

SEQ ID NO: 6 - protein, 5 aa, synthetic construct
MRSPA